European Patent Application EP 4 163 393 A1, published April 12, 2023. Title: PREDICTION OF THERAPEUTIC RESPONSE IN INFLAMMATORY CONDITIONS. Applicant: Liquid Bioscience, Inc. The sequence listing filed with the application follows.

SEQUENCE LISTING (5 sequences)

SEQ ID NO: 1 - DNA, 344 bp, Homo sapiens
  source 1..344: mol_type = genomic DNA
gaagctccttagtgaggagctgccatgctgggccatccaccatctggattcctacgactcagggaatagaacactgcaccttccagaagcacttgtttcttcgtgggtacaccaccagctgagaaagaagcctcatgatgattgttgtcttatggatgcttctcattgcaggaaccatgtggaagggatataaatatcccccaggagggactccagtggaagtaagcaaggatgatcctggtgaagtaatgcagctgtgaagctcacctgaccagctgtacagttcctgttgttggtttcacataaagtaattgcacattattttgtcataaaaaaaaaaaaaa

SEQ ID NO: 2 - DNA, 985 bp, Homo sapiens
  source 1..985: mol_type = genomic DNA
atgtaaatcacacagatgttggtagagaaaaaggcatactggtattgaaactgtaaactggcctgtttacttcgtctcctaacaaaaaacactttggattcaggttctccacagcagtcttccactggccacagtgaggggagctaggtttccccagtctccagctagaaaaactcagaacatctaaagatctgaaagatggaaaaaagagaactaaaggcttctgttccaaaatttgacaagattccttggcttagtgaggccagccttgtaaacaagccattagtgctcagccttcccagaagatatcctcatacctctgcgacttttctgacttcatccaagaagaatatgaatttgccaattttgtttcaagttccagatgttttatctaaggccaggaggaaccagtgtgactccatgctgctcagaaaccaacagctgtgctccacatgtcaagaaatgaaaatggtacaaccaagaacaatgaaaatcccagatgatccaaaagcatcctttgagaattgtatgagttatagaatgagtcttcatcaacccaaattccagactacacctgagcctttccatgatgacatcccaacagaaagcattcactacagactgcccattctgggccccaggacagctgtcttccacggattactgacagaggcctacaaaactctaaaagagagacaacgttcttccttgcccagaaaggaaccaataggcaagacaacgaggcagtgagcggtaggagctcatcacctcccagactcccagagagaaaataacctcgccaagccaatctttgacactggcaccttctcctcacaattttctctcttctcccaaaagatgatttaattttgccttcctaagattgctggtattctagctcttacctctatgttctttctcacgtctcctaaagacaaaattgtttaatttacatgattataaagatctgtttatgaaaatggaa

SEQ ID NO: 3 - DNA, 722 bp, Homo sapiens
  source 1..722: mol_type = genomic DNA
ttttttttttttttttttagcaaaagctttcagtctttatttacagtatatagaaggttactgttttcattttaggtggaagagtctgatcagtaggaacaccccagaggaaggacatctttagcgatagaatttacataccgttagctcacagtaattgattagtagcagggctctgtagtacagagctagctgggcatgttatttgggatgtctttgatgctgtggttttccgaagcttgctggctgcatgcttgttgcctttgttcgtgacacaggtaattacttgataaaatgaagtgcatcgctgtgaacaattgaccctttggaacaatccaggctggtcagcagtctaaagccacactttaaagccatcatgatagcctcaaacttaagagtttccaaggtacagacaaaggtgttgtcttcctttagtacaagtcgagtgccattttcagactttatgaagtatttaaattggatgatatttgacgatattgaaaactcctctggaaatccatccagcctgcttttggacaccagaacaatgcgagactttatttttgatatgaaatcaggagcattacagaagattcttaatccttgtgaacgatcgtggttatctgttatttccaagaaagtagtctctctgggtgttagctgttctttctcccacctggatntcacttcctctgccagtcncttgagctgaaagattctgc

SEQ ID NO: 4 - protein, 586 aa, Human herpesvirus 5
MPRVDPNLRNRARRPRARRGGGGGVGSNSSRHSGKCRRQRRALSAPPLTFLATTTTTTMMGVASTDDDSLLLKTPDELDKYSGSPQTILTLTDKHDIRQPRVHRGTYHLIQLHLDLRPEELRDPFQILLSTPLQLGEANDESQTAPATLQEEETAASHEPEKKKEKQEKKEEDEDDRNDDRERGILCVVSNEDSDVRPAFSLFPARPGCHILRSVIDQQLTRMAIVRLSLNLFALRIITPLLKRLPLRRKAAHHTALHDCLALHLPELTFEPTLDINNVTENAASVADTAESTDADLTPTLTVRVRHALCWHRVEGGISGPRGLTSRISARLSETTAKTLGPSVFGRLELDPNESPPDLTLSSLTLYQDGILRFNVTCDRTEAPADPVAFRLRLRRETVRRPFFSDAPLPYFVPPRSGAADEGLEVRVPYELTLKNSHTLRIYRRFYGPYLGVFVPHNRQGLKMPVTVWLPRSWLELTVLVSDENGATFPRDALLGRLYFISSKHTLNRGCLSAMTHQVKSTLHSRSTSHSPSQQQLSVLGASIALEDLLPMRLASPETEPQDCKLTENTTEKTSPVTLAMVCGDL

SEQ ID NO: 5 - DNA, 144 bp, Homo sapiens
  source 1..144: mol_type = genomic DNA
ggaaccaatccaaatgcccatcaatgatagactagataaagaaaatatagtacatatgcaccatgtaatactatgcagccgtaaaaaaaaaaaaaaaaaaagacagacaaggccaaggccaggcacggtgggtaaaaaaaaaaa